European Patent Application EP 4 144 754 A1, published March 8, 2023. Title: Variant of D-allulose 3-epimerase, manufacturing method thereof and manufacturing method of D-alluose using the same. Applicant: DAESANG CORPORATION. The sequence listing filed with the application follows.

SEQUENCE LISTING (26 sequences)

SEQ ID NO: 1 - protein, 294 aa, Unknown
  Wild type D-allulose 3-epimerase derived from Flavonifractor plautii
MNPIGMHYGFWSHNWDEIAYIPLMEKLAWLGFDICEVASAEWGYYDDARLRELKACADHNGLGITYSIGLEAKYDLASDDPAVRENGIRHVTRILESMPKVGAAILNGVSYAGWQALPDHGITLDEKRRKEELALESMSRLMKVAEDCGVLYCCEVVNRFEQYLLNTAKEGVEFVKRLGSPNARVLLDTFHMNIEEDSMVDAILEAGPWLGHFHVGENNRRPAGSTNRLPWKDMAAALKQVNYQGAIVMEPFVLMGGTIPYDIKVWRDLSGGAGEAGLDEMAGRACRFLKELTA

SEQ ID NO: 2 - protein, 294 aa, Artificial Sequence
  D-allulose 3-epimerase variant W29K
MNPIGMHYGFWSHNWDEIAYIPLMEKLAKLGFDICEVASAEWGYYDDARLRELKACADHNGLGITYSIGLEAKYDLASDDPAVRENGIRHVTRILESMPKVGAAILNGVSYAGWQALPDHGITLDEKRRKEELALESMSRLMKVAEDCGVLYCCEVVNRFEQYLLNTAKEGVEFVKRLGSPNARVLLDTFHMNIEEDSMVDAILEAGPWLGHFHVGENNRRPAGSTNRLPWKDMAAALKQVNYQGAIVMEPFVLMGGTIPYDIKVWRDLSGGAGEAGLDEMAGRACRFLKELTA

SEQ ID NO: 3 - protein, 294 aa, Artificial Sequence
  D-allulose 3-epimerase variant C35L
MNPIGMHYGFWSHNWDEIAYIPLMEKLAWLGFDILEVASAEWGYYDDARLRELKACADHNGLGITYSIGLEAKYDLASDDPAVRENGIRHVTRILESMPKVGAAILNGVSYAGWQALPDHGITLDEKRRKEELALESMSRLMKVAEDCGVLYCCEVVNRFEQYLLNTAKEGVEFVKRLGSPNARVLLDTFHMNIEEDSMVDAILEAGPWLGHFHVGENNRRPAGSTNRLPWKDMAAALKQVNYQGAIVMEPFVLMGGTIPYDIKVWRDLSGGAGEAGLDEMAGRACRFLKELTA

SEQ ID NO: 4 - protein, 294 aa, Artificial Sequence
  D-allulose 3-epimerase variant D79P
MNPIGMHYGFWSHNWDEIAYIPLMEKLAWLGFDICEVASAEWGYYDDARLRELKACADHNGLGITYSIGLEAKYDLASPDPAVRENGIRHVTRILESMPKVGAAILNGVSYAGWQALPDHGITLDEKRRKEELALESMSRLMKVAEDCGVLYCCEVVNRFEQYLLNTAKEGVEFVKRLGSPNARVLLDTFHMNIEEDSMVDAILEAGPWLGHFHVGENNRRPAGSTNRLPWKDMAAALKQVNYQGAIVMEPFVLMGGTIPYDIKVWRDLSGGAGEAGLDEMAGRACRFLKELTA

SEQ ID NO: 5 - protein, 294 aa, Artificial Sequence
  D-allulose 3-epimerase variant V109A
MNPIGMHYGFWSHNWDEIAYIPLMEKLAWLGFDICEVASAEWGYYDDARLRELKACADHNGLGITYSIGLEAKYDLASDDPAVRENGIRHVTRILESMPKVGAAILNGASYAGWQALPDHGITLDEKRRKEELALESMSRLMKVAEDCGVLYCCEVVNRFEQYLLNTAKEGVEFVKRLGSPNARVLLDTFHMNIEEDSMVDAILEAGPWLGHFHVGENNRRPAGSTNRLPWKDMAAALKQVNYQGAIVMEPFVLMGGTIPYDIKVWRDLSGGAGEAGLDEMAGRACRFLKELTA

SEQ ID NO: 6 - protein, 294 aa, Artificial Sequence
  D-allulose 3-epimerase variant M199F
MNPIGMHYGFWSHNWDEIAYIPLMEKLAWLGFDICEVASAEWGYYDDARLRELKACADHNGLGITYSIGLEAKYDLASDDPAVRENGIRHVTRILESMPKVGAAILNGVSYAGWQALPDHGITLDEKRRKEELALESMSRLMKVAEDCGVLYCCEVVNRFEQYLLNTAKEGVEFVKRLGSPNARVLLDTFHMNIEEDSFVDAILEAGPWLGHFHVGENNRRPAGSTNRLPWKDMAAALKQVNYQGAIVMEPFVLMGGTIPYDIKVWRDLSGGAGEAGLDEMAGRACRFLKELTA

SEQ ID NO: 7 - protein, 294 aa, Artificial Sequence
  D-allulose 3-epimerase variant G216S
MNPIGMHYGFWSHNWDEIAYIPLMEKLAWLGFDICEVASAEWGYYDDARLRELKACADHNGLGITYSIGLEAKYDLASDDPAVRENGIRHVTRILESMPKVGAAILNGVSYAGWQALPDHGITLDEKRRKEELALESMSRLMKVAEDCGVLYCCEVVNRFEQYLLNTAKEGVEFVKRLGSPNARVLLDTFHMNIEEDSMVDAILEAGPWLGHFHVSENNRRPAGSTNRLPWKDMAAALKQVNYQGAIVMEPFVLMGGTIPYDIKVWRDLSGGAGEAGLDEMAGRACRFLKELTA

SEQ ID NO: 8 - protein, 294 aa, Artificial Sequence
  D-allulose 3-epimerase variant N218C
MNPIGMHYGFWSHNWDEIAYIPLMEKLAWLGFDICEVASAEWGYYDDARLRELKACADHNGLGITYSIGLEAKYDLASDDPAVRENGIRHVTRILESMPKVGAAILNGVSYAGWQALPDHGITLDEKRRKEELALESMSRLMKVAEDCGVLYCCEVVNRFEQYLLNTAKEGVEFVKRLGSPNARVLLDTFHMNIEEDSMVDAILEAGPWLGHFHVGECNRRPAGSTNRLPWKDMAAALKQVNYQGAIVMEPFVLMGGTIPYDIKVWRDLSGGAGEAGLDEMAGRACRFLKELTA

SEQ ID NO: 9 - protein, 294 aa, Artificial Sequence
  D-allulose 3-epimerase variant M234I
MNPIGMHYGFWSHNWDEIAYIPLMEKLAWLGFDICEVASAEWGYYDDARLRELKACADHNGLGITYSIGLEAKYDLASDDPAVRENGIRHVTRILESMPKVGAAILNGVSYAGWQALPDHGITLDEKRRKEELALESMSRLMKVAEDCGVLYCCEVVNRFEQYLLNTAKEGVEFVKRLGSPNARVLLDTFHMNIEEDSMVDAILEAGPWLGHFHVGENNRRPAGSTNRLPWKDIAAALKQVNYQGAIVMEPFVLMGGTIPYDIKVWRDLSGGAGEAGLDEMAGRACRFLKELTA

SEQ ID NO: 10 - protein, 294 aa, Artificial Sequence
  D-allulose 3-epimerase variant W29K/G216S
MNPIGMHYGFWSHNWDEIAYIPLMEKLAKLGFDICEVASAEWGYYDDARLRELKACADHNGLGITYSIGLEAKYDLASDDPAVRENGIRHVTRILESMPKVGAAILNGVSYAGWQALPDHGITLDEKRRKEELALESMSRLMKVAEDCGVLYCCEVVNRFEQYLLNTAKEGVEFVKRLGSPNARVLLDTFHMNIEEDSMVDAILEAGPWLGHFHVSENNRRPAGSTNRLPWKDMAAALKQVNYQGAIVMEPFVLMGGTIPYDIKVWRDLSGGAGEAGLDEMAGRACRFLKELTA

SEQ ID NO: 11 - protein, 294 aa, Artificial Sequence
  D-allulose 3-epimerase variant W29K/M234I
MNPIGMHYGFWSHNWDEIAYIPLMEKLAKLGFDICEVASAEWGYYDDARLRELKACADHNGLGITYSIGLEAKYDLASDDPAVRENGIRHVTRILESMPKVGAAILNGVSYAGWQALPDHGITLDEKRRKEELALESMSRLMKVAEDCGVLYCCEVVNRFEQYLLNTAKEGVEFVKRLGSPNARVLLDTFHMNIEEDSMVDAILEAGPWLGHFHVGENNRRPAGSTNRLPWKDIAAALKQVNYQGAIVMEPFVLMGGTIPYDIKVWRDLSGGAGEAGLDEMAGRACRFLKELTA

SEQ ID NO: 12 - protein, 294 aa, Artificial Sequence
  D-allulose 3-epimerase variant G216S/M234I
MNPIGMHYGFWSHNWDEIAYIPLMEKLAWLGFDICEVASAEWGYYDDARLRELKACADHNGLGITYSIGLEAKYDLASDDPAVRENGIRHVTRILESMPKVGAAILNGVSYAGWQALPDHGITLDEKRRKEELALESMSRLMKVAEDCGVLYCCEVVNRFEQYLLNTAKEGVEFVKRLGSPNARVLLDTFHMNIEEDSMVDAILEAGPWLGHFHVSENNRRPAGSTNRLPWKDIAAALKQVNYQGAIVMEPFVLMGGTIPYDIKVWRDLSGGAGEAGLDEMAGRACRFLKELTA

SEQ ID NO: 13 - protein, 294 aa, Artificial Sequence
  D-allulose 3-epimerase variant W29K/G216S/M234I
MNPIGMHYGFWSHNWDEIAYIPLMEKLAKLGFDICEVASAEWGYYDDARLRELKACADHNGLGITYSIGLEAKYDLASDDPAVRENGIRHVTRILESMPKVGAAILNGVSYAGWQALPDHGITLDEKRRKEELALESMSRLMKVAEDCGVLYCCEVVNRFEQYLLNTAKEGVEFVKRLGSPNARVLLDTFHMNIEEDSMVDAILEAGPWLGHFHVSENNRRPAGSTNRLPWKDIAAALKQVNYQGAIVMEPFVLMGGTIPYDIKVWRDLSGGAGEAGLDEMAGRACRFLKELTA

SEQ ID NO: 14 - DNA, 885 bp, Unknown
  Polynucleotide coding wild type D-allulose 3-epimerase derived from Flavonifractor plautii
atgaacccgattggaatgcactacggcttctggagccacaactgggacgagattgcatacatacccctgatggagaagctggcctggctgggctttgacatctgcgaggtggcctccgccgagtggggctattacgacgacgccaggctgcgggagctgaaggcctgcgccgatcacaacggcctgggcatcacctattccatcggcctggaggccaaatacgacctggccagcgacgatccggcggtgcgggagaacggcatccgccatgtcacccgcatcctggagagcatgcccaaggtgggggcggccatcctcaacggcgtgtcctacgccgggtggcaggccctgcccgaccacggaatcaccctggacgagaagcgccgcaaggaggagcttgccctggagtccatgtcccggctcatgaaggtggcggaggactgcggcgtgctctactgctgcgaggtggtcaaccgcttcgagcagtacctgctcaacaccgccaaagagggcgtggagtttgtcaagcgcctgggcagtcccaacgcccgggtgctgctggataccttccacatgaacatcgaggaggacagcatggtggacgccattctggaggcgggcccctggctggggcatttccacgtgggggagaacaaccgccgccccgccggctccaccaaccgcctgccctggaaggacatggccgccgccctcaagcaggtgaactaccagggggccattgtgatggagcccttcgtgctcatggggggtaccattccctatgatatcaaggtctggcgggatctcagcggcggggccggggaggccgggctggacgagatggcgggccgggcctgccggttcctcaaggagctgaccgcgtaa

SEQ ID NO: 15 - DNA, 885 bp, Artificial Sequence
  Polynucleotide coding D-allulose 3-epimerase variant W29K
atgaacccgattggaatgcactacggcttctggagccacaactgggacgagattgcatacatacccctgatggagaagctggccaaactgggctttgacatctgcgaggtggcctccgccgagtggggctattacgacgacgccaggctgcgggagctgaaggcctgcgccgatcacaacggcctgggcatcacctattccatcggcctggaggccaaatacgacctggccagcgacgatccggcggtgcgggagaacggcatccgccatgtcacccgcatcctggagagcatgcccaaggtgggggcggccatcctcaacggcgtgtcctacgccgggtggcaggccctgcccgaccacggaatcaccctggacgagaagcgccgcaaggaggagcttgccctggagtccatgtcccggctcatgaaggtggcggaggactgcggcgtgctctactgctgcgaggtggtcaaccgcttcgagcagtacctgctcaacaccgccaaagagggcgtggagtttgtcaagcgcctgggcagtcccaacgcccgggtgctgctggataccttccacatgaacatcgaggaggacagcatggtggacgccattctggaggcgggcccctggctggggcatttccacgtgggggagaacaaccgccgccccgccggctccaccaaccgcctgccctggaaggacatggccgccgccctcaagcaggtgaactaccagggggccattgtgatggagcccttcgtgctcatggggggtaccattccctatgatatcaaggtctggcgggatctcagcggcggggccggggaggccgggctggacgagatggcgggccgggcctgccggttcctcaaggagctgaccgcgtaa

SEQ ID NO: 16 - DNA, 885 bp, Artificial Sequence
  Polynucleotide coding D-allulose 3-epimerase variant C35L
atgaacccgattggaatgcactacggcttctggagccacaactgggacgagattgcatacatacccctgatggagaagctggcctggctgggctttgacatcctggaggtggcctccgccgagtggggctattacgacgacgccaggctgcgggagctgaaggcctgcgccgatcacaacggcctgggcatcacctattccatcggcctggaggccaaatacgacctggccagcgacgatccggcggtgcgggagaacggcatccgccatgtcacccgcatcctggagagcatgcccaaggtgggggcggccatcctcaacggcgtgtcctacgccgggtggcaggccctgcccgaccacggaatcaccctggacgagaagcgccgcaaggaggagcttgccctggagtccatgtcccggctcatgaaggtggcggaggactgcggcgtgctctactgctgcgaggtggtcaaccgcttcgagcagtacctgctcaacaccgccaaagagggcgtggagtttgtcaagcgcctgggcagtcccaacgcccgggtgctgctggataccttccacatgaacatcgaggaggacagcatggtggacgccattctggaggcgggcccctggctggggcatttccacgtgggggagaacaaccgccgccccgccggctccaccaaccgcctgccctggaaggacatggccgccgccctcaagcaggtgaactaccagggggccattgtgatggagcccttcgtgctcatggggggtaccattccctatgatatcaaggtctggcgggatctcagcggcggggccggggaggccgggctggacgagatggcgggccgggcctgccggttcctcaaggagctgaccgcgtaa

SEQ ID NO: 17 - DNA, 885 bp, Artificial Sequence
  Polynucleotide coding D-allulose 3-epimerase variant D79P
atgaacccgattggaatgcactacggcttctggagccacaactgggacgagattgcatacatacccctgatggagaagctggcctggctgggctttgacatctgcgaggtggcctccgccgagtggggctattacgacgacgccaggctgcgggagctgaaggcctgcgccgatcacaacggcctgggcatcacctattccatcggcctggaggccaaatacgacctggccagccccgatccggcggtgcgggagaacggcatccgccatgtcacccgcatcctggagagcatgcccaaggtgggggcggccatcctcaacggcgtgtcctacgccgggtggcaggccctgcccgaccacggaatcaccctggacgagaagcgccgcaaggaggagcttgccctggagtccatgtcccggctcatgaaggtggcggaggactgcggcgtgctctactgctgcgaggtggtcaaccgcttcgagcagtacctgctcaacaccgccaaagagggcgtggagtttgtcaagcgcctgggcagtcccaacgcccgggtgctgctggataccttccacatgaacatcgaggaggacagcatggtggacgccattctggaggcgggcccctggctggggcatttccacgtgggggagaacaaccgccgccccgccggctccaccaaccgcctgccctggaaggacatggccgccgccctcaagcaggtgaactaccagggggccattgtgatggagcccttcgtgctcatggggggtaccattccctatgatatcaaggtctggcgggatctcagcggcggggccggggaggccgggctggacgagatggcgggccgggcctgccggttcctcaaggagctgaccgcgtaa

SEQ ID NO: 18 - DNA, 885 bp, Artificial Sequence
  Polynucleotide coding D-allulose 3-epimerase variant V109A
atgaacccgattggaatgcactacggcttctggagccacaactgggacgagattgcatacatacccctgatggagaagctggcctggctgggctttgacatctgcgaggtggcctccgccgagtggggctattacgacgacgccaggctgcgggagctgaaggcctgcgccgatcacaacggcctgggcatcacctattccatcggcctggaggccaaatacgacctggccagcgacgatccggcggtgcgggagaacggcatccgccatgtcacccgcatcctggagagcatgcccaaggtgggggcggccatcctcaacggcgcctcctacgccgggtggcaggccctgcccgaccacggaatcaccctggacgagaagcgccgcaaggaggagcttgccctggagtccatgtcccggctcatgaaggtggcggaggactgcggcgtgctctactgctgcgaggtggtcaaccgcttcgagcagtacctgctcaacaccgccaaagagggcgtggagtttgtcaagcgcctgggcagtcccaacgcccgggtgctgctggataccttccacatgaacatcgaggaggacagcatggtggacgccattctggaggcgggcccctggctggggcatttccacgtgggggagaacaaccgccgccccgccggctccaccaaccgcctgccctggaaggacatggccgccgccctcaagcaggtgaactaccagggggccattgtgatggagcccttcgtgctcatggggggtaccattccctatgatatcaaggtctggcgggatctcagcggcggggccggggaggccgggctggacgagatggcgggccgggcctgccggttcctcaaggagctgaccgcgtaa

SEQ ID NO: 19 - DNA, 885 bp, Artificial Sequence
  Polynucleotide coding D-allulose 3-epimerase variant M199F
atgaacccgattggaatgcactacggcttctggagccacaactgggacgagattgcatacatacccctgatggagaagctggcctggctgggctttgacatctgcgaggtggcctccgccgagtggggctattacgacgacgccaggctgcgggagctgaaggcctgcgccgatcacaacggcctgggcatcacctattccatcggcctggaggccaaatacgacctggccagcgacgatccggcggtgcgggagaacggcatccgccatgtcacccgcatcctggagagcatgcccaaggtgggggcggccatcctcaacggcgtgtcctacgccgggtggcaggccctgcccgaccacggaatcaccctggacgagaagcgccgcaaggaggagcttgccctggagtccatgtcccggctcatgaaggtggcggaggactgcggcgtgctctactgctgcgaggtggtcaaccgcttcgagcagtacctgctcaacaccgccaaagagggcgtggagtttgtcaagcgcctgggcagtcccaacgcccgggtgctgctggataccttccacatgaacatcgaggaggacagcttcgtggacgccattctggaggcgggcccctggctggggcatttccacgtgggggagaacaaccgccgccccgccggctccaccaaccgcctgccctggaaggacatggccgccgccctcaagcaggtgaactaccagggggccattgtgatggagcccttcgtgctcatggggggtaccattccctatgatatcaaggtctggcgggatctcagcggcggggccggggaggccgggctggacgagatggcgggccgggcctgccggttcctcaaggagctgaccgcgtaa

SEQ ID NO: 20 - DNA, 885 bp, Artificial Sequence
  Polynucleotide coding D-allulose 3-epimerase variant G216S
atgaacccgattggaatgcactacggcttctggagccacaactgggacgagattgcatacatacccctgatggagaagctggcctggctgggctttgacatctgcgaggtggcctccgccgagtggggctattacgacgacgccaggctgcgggagctgaaggcctgcgccgatcacaacggcctgggcatcacctattccatcggcctggaggccaaatacgacctggccagcgacgatccggcggtgcgggagaacggcatccgccatgtcacccgcatcctggagagcatgcccaaggtgggggcggccatcctcaacggcgtgtcctacgccgggtggcaggccctgcccgaccacggaatcaccctggacgagaagcgccgcaaggaggagcttgccctggagtccatgtcccggctcatgaaggtggcggaggactgcggcgtgctctactgctgcgaggtggtcaaccgcttcgagcagtacctgctcaacaccgccaaagagggcgtggagtttgtcaagcgcctgggcagtcccaacgcccgggtgctgctggataccttccacatgaacatcgaggaggacagcatggtggacgccattctggaggcgggcccctggctggggcatttccacgtgagcgagaacaaccgccgccccgccggctccaccaaccgcctgccctggaaggacatggccgccgccctcaagcaggtgaactaccagggggccattgtgatggagcccttcgtgctcatggggggtaccattccctatgatatcaaggtctggcgggatctcagcggcggggccggggaggccgggctggacgagatggcgggccgggcctgccggttcctcaaggagctgaccgcgtaa

SEQ ID NO: 21 - DNA, 885 bp, Artificial Sequence
  Polynucleotide coding D-allulose 3-epimerase variant N218C
atgaacccgattggaatgcactacggcttctggagccacaactgggacgagattgcatacatacccctgatggagaagctggcctggctgggctttgacatctgcgaggtggcctccgccgagtggggctattacgacgacgccaggctgcgggagctgaaggcctgcgccgatcacaacggcctgggcatcacctattccatcggcctggaggccaaatacgacctggccagcgacgatccggcggtgcgggagaacggcatccgccatgtcacccgcatcctggagagcatgcccaaggtgggggcggccatcctcaacggcgtgtcctacgccgggtggcaggccctgcccgaccacggaatcaccctggacgagaagcgccgcaaggaggagcttgccctggagtccatgtcccggctcatgaaggtggcggaggactgcggcgtgctctactgctgcgaggtggtcaaccgcttcgagcagtacctgctcaacaccgccaaagagggcgtggagtttgtcaagcgcctgggcagtcccaacgcccgggtgctgctggataccttccacatgaacatcgaggaggacagcatggtggacgccattctggaggcgggcccctggctggggcatttccacgtgggggagtgcaaccgccgccccgccggctccaccaaccgcctgccctggaaggacatggccgccgccctcaagcaggtgaactaccagggggccattgtgatggagcccttcgtgctcatggggggtaccattccctatgatatcaaggtctggcgggatctcagcggcggggccggggaggccgggctggacgagatggcgggccgggcctgccggttcctcaaggagctgaccgcgtaa

SEQ ID NO: 22 - DNA, 885 bp, Artificial Sequence
  Polynucleotide coding D-allulose 3-epimerase variant M234I
atgaacccgattggaatgcactacggcttctggagccacaactgggacgagattgcatacatacccctgatggagaagctggcctggctgggctttgacatctgcgaggtggcctccgccgagtggggctattacgacgacgccaggctgcgggagctgaaggcctgcgccgatcacaacggcctgggcatcacctattccatcggcctggaggccaaatacgacctggccagcgacgatccggcggtgcgggagaacggcatccgccatgtcacccgcatcctggagagcatgcccaaggtgggggcggccatcctcaacggcgtgtcctacgccgggtggcaggccctgcccgaccacggaatcaccctggacgagaagcgccgcaaggaggagcttgccctggagtccatgtcccggctcatgaaggtggcggaggactgcggcgtgctctactgctgcgaggtggtcaaccgcttcgagcagtacctgctcaacaccgccaaagagggcgtggagtttgtcaagcgcctgggcagtcccaacgcccgggtgctgctggataccttccacatgaacatcgaggaggacagcatggtggacgccattctggaggcgggcccctggctggggcatttccacgtgggggagaacaaccgccgccccgccggctccaccaaccgcctgccctggaaggacattgccgccgccctcaagcaggtgaactaccagggggccattgtgatggagcccttcgtgctcatggggggtaccattccctatgatatcaaggtctggcgggatctcagcggcggggccggggaggccgggctggacgagatggcgggccgggcctgccggttcctcaaggagctgaccgcgtaa

SEQ ID NO: 23 - DNA, 885 bp, Artificial Sequence
  Polynucleotide coding D-allulose 3-epimerase variant W29K/G216S
atgaacccgattggaatgcactacggcttctggagccacaactgggacgagattgcatacatacccctgatggagaagctggccaaactgggctttgacatctgcgaggtggcctccgccgagtggggctattacgacgacgccaggctgcgggagctgaaggcctgcgccgatcacaacggcctgggcatcacctattccatcggcctggaggccaaatacgacctggccagcgacgatccggcggtgcgggagaacggcatccgccatgtcacccgcatcctggagagcatgcccaaggtgggggcggccatcctcaacggcgtgtcctacgccgggtggcaggccctgcccgaccacggaatcaccctggacgagaagcgccgcaaggaggagcttgccctggagtccatgtcccggctcatgaaggtggcggaggactgcggcgtgctctactgctgcgaggtggtcaaccgcttcgagcagtacctgctcaacaccgccaaagagggcgtggagtttgtcaagcgcctgggcagtcccaacgcccgggtgctgctggataccttccacatgaacatcgaggaggacagcatggtggacgccattctggaggcgggcccctggctggggcatttccacgtgagcgagaacaaccgccgccccgccggctccaccaaccgcctgccctggaaggacatggccgccgccctcaagcaggtgaactaccagggggccattgtgatggagcccttcgtgctcatggggggtaccattccctatgatatcaaggtctggcgggatctcagcggcggggccggggaggccgggctggacgagatggcgggccgggcctgccggttcctcaaggagctgaccgcgtaa

SEQ ID NO: 24 - DNA, 885 bp, Artificial Sequence
  Polynucleotide coding D-allulose 3-epimerase variant W29K/M234I
atgaacccgattggaatgcactacggcttctggagccacaactgggacgagattgcatacatacccctgatggagaagctggccaaactgggctttgacatctgcgaggtggcctccgccgagtggggctattacgacgacgccaggctgcgggagctgaaggcctgcgccgatcacaacggcctgggcatcacctattccatcggcctggaggccaaatacgacctggccagcgacgatccggcggtgcgggagaacggcatccgccatgtcacccgcatcctggagagcatgcccaaggtgggggcggccatcctcaacggcgtgtcctacgccgggtggcaggccctgcccgaccacggaatcaccctggacgagaagcgccgcaaggaggagcttgccctggagtccatgtcccggctcatgaaggtggcggaggactgcggcgtgctctactgctgcgaggtggtcaaccgcttcgagcagtacctgctcaacaccgccaaagagggcgtggagtttgtcaagcgcctgggcagtcccaacgcccgggtgctgctggataccttccacatgaacatcgaggaggacagcatggtggacgccattctggaggcgggcccctggctggggcatttccacgtgggggagaacaaccgccgccccgccggctccaccaaccgcctgccctggaaggacattgccgccgccctcaagcaggtgaactaccagggggccattgtgatggagcccttcgtgctcatggggggtaccattccctatgatatcaaggtctggcgggatctcagcggcggggccggggaggccgggctggacgagatggcgggccgggcctgccggttcctcaaggagctgaccgcgtaa

SEQ ID NO: 25 - DNA, 885 bp, Artificial Sequence
  Polynucleotide coding D-allulose 3-epimerase variant G216S/M234I
atgaacccgattggaatgcactacggcttctggagccacaactgggacgagattgcatacatacccctgatggagaagctggcctggctgggctttgacatctgcgaggtggcctccgccgagtggggctattacgacgacgccaggctgcgggagctgaaggcctgcgccgatcacaacggcctgggcatcacctattccatcggcctggaggccaaatacgacctggccagcgacgatccggcggtgcgggagaacggcatccgccatgtcacccgcatcctggagagcatgcccaaggtgggggcggccatcctcaacggcgtgtcctacgccgggtggcaggccctgcccgaccacggaatcaccctggacgagaagcgccgcaaggaggagcttgccctggagtccatgtcccggctcatgaaggtggcggaggactgcggcgtgctctactgctgcgaggtggtcaaccgcttcgagcagtacctgctcaacaccgccaaagagggcgtggagtttgtcaagcgcctgggcagtcccaacgcccgggtgctgctggataccttccacatgaacatcgaggaggacagcatggtggacgccattctggaggcgggcccctggctggggcatttccacgtgagcgagaacaaccgccgccccgccggctccaccaaccgcctgccctggaaggacattgccgccgccctcaagcaggtgaactaccagggggccattgtgatggagcccttcgtgctcatggggggtaccattccctatgatatcaaggtctggcgggatctcagcggcggggccggggaggccgggctggacgagatggcgggccgggcctgccggttcctcaaggagctgaccgcgtaa

SEQ ID NO: 26 - DNA, 885 bp, Artificial Sequence
  Polynucleotide coding D-allulose 3-epimerase variant W29K/G216S/M234I
atgaacccgattggaatgcactacggcttctggagccacaactgggacgagattgcatacatacccctgatggagaagctggccaaactgggctttgacatctgcgaggtggcctccgccgagtggggctattacgacgacgccaggctgcgggagctgaaggcctgcgccgatcacaacggcctgggcatcacctattccatcggcctggaggccaaatacgacctggccagcgacgatccggcggtgcgggagaacggcatccgccatgtcacccgcatcctggagagcatgcccaaggtgggggcggccatcctcaacggcgtgtcctacgccgggtggcaggccctgcccgaccacggaatcaccctggacgagaagcgccgcaaggaggagcttgccctggagtccatgtcccggctcatgaaggtggcggaggactgcggcgtgctctactgctgcgaggtggtcaaccgcttcgagcagtacctgctcaacaccgccaaagagggcgtggagtttgtcaagcgcctgggcagtcccaacgcccgggtgctgctggataccttccacatgaacatcgaggaggacagcatggtggacgccattctggaggcgggcccctggctggggcatttccacgtgagcgagaacaaccgccgccccgccggctccaccaaccgcctgccctggaaggacattgccgccgccctcaagcaggtgaactaccagggggccattgtgatggagcccttcgtgctcatggggggtaccattccctatgatatcaaggtctggcgggatctcagcggcggggccggggaggccgggctggacgagatggcgggccgggcctgccggttcctcaaggagctgaccgcgtaa